European Patent Application EP 4 186 921 A1, published May 31, 2023. Title: Gene editing for autosomal dominant diseases. Applicant: The Trustees of Columbia University in the City of New York. The sequence listing filed with the application follows.

SEQUENCE LISTING (49 sequences)

SEQ ID NO: 1 - DNA, 20 bp, Homo sapiens
  source 1..20: mol_type = other DNA
ggacggtgacgtagagcgtg

SEQ ID NO: 2 - DNA, 20 bp, Homo sapiens
  source 1..20: mol_type = other DNA
gacgaagtatccatgcagag

SEQ ID NO: 3 - DNA, 20 bp, Homo sapiens
  source 1..20: mol_type = other DNA
tgagaccacaaatgaatgct

SEQ ID NO: 4 - DNA, 22 bp, Mus musculus
  source 1..22: mol_type = other DNA
aactactacacactcaagcctg

SEQ ID NO: 5 - DNA, 20 bp, Mus musculus
  source 1..20: mol_type = other DNA
gtagtactgcggctgctcga

SEQ ID NO: 6 - DNA, 20 bp, Mus musculus
  source 1..20: mol_type = other DNA
gctcatgctgccggcgattc

SEQ ID NO: 7 - DNA, 20 bp, Drosophila melanogaster
  source 1..20: mol_type = other DNA
ggttttggacaatggaaccg

SEQ ID NO: 8 - DNA, 1047 bp, Homo sapiens
  source 1..1047: mol_type = other DNA
atgaatggcacagaaggccctaacttctacgtgcccttctccaatgcgacgggtgtggtacgcagccccttcgagtacccacagtactacctggctgagccatggcagttctccatgctggccgcctacatgtttctgctgatcgtgctgggcttccccatcaacttcctcacgctctacgtcaccgtccagcacaagaagctgcgcacgcctctcaactacatcctgctcaacctagccgtggctgacctcttcatggtcctaggtggcttcaccagcaccctctacacctctctgcatggatacttcgtcttcgggcccacaggatgcaatttggagggcttctttgccaccctgggcggtgaaattgccctgtggtccttggtggtcctggccatcgagcggtacgtggtggtgtgtaagcccatgagcaacttccgcttcggggagaaccatgccatcatgggcgttgccttcacctgggtcatggcgctggcctgcgccgcacccccactcgccggctggtccaggtacatccccgagggcctgcagtgctcgtgtggaatcgactactacacgctcaagccggaggtcaacaacgagtcttttgtcatctacatgttcgtggtccacttcaccatccccatgattatcatctttttctgctatgggcagctcgtcttcaccgtcaaggaggccgctgcccagcagcaggagtcagccaccacacagaaggcagagaaggaggtcacccgcatggtcatcatcatggtcatcgctttcctgatctgctgggtgccctacgccagcgtggcattctacatcttcacccaccagggctccaacttcggtcccatcttcatgaccatcccagcgttctttgccaagagcgccgccatctacaaccctgtcatctatatcatgatgaacaagcagttccggaactgcatgctcaccaccatctgctgcggcaagaacccactgggtgacgatgaggcctctgctaccgtgtccaagacggagacgagccaggtggccccggcctaa

SEQ ID NO: 9 - DNA, 1044 bp, Homo sapiens
  source 1..1044: mol_type = other DNA
atgaatggcacagaaggccctaacttctacgtgcccttctccaatgcgacgggtgtggtacgcagccccttcgagtacccacagtactacctggctgagccatggcagttctccatgctggccgcctacatgtttctgctgatcgtgctgggcttccccatcaactttcttacactgtacgtcaccgtccagcacaagaagctgcgcacgcctctcaactacatcctgctcaacctagccgtggctgacctcttcatggtcctaggtggcttcaccagcaccctctacacgtcgcttcacggatatttcgtcttcgggcccacaggatgcaatttggagggcttctttgccaccctgggcggtgaaattgccctgtggtccttggtggtcctggccatcgagcggtacgtggtggtgtgtaagcccatgagcaacttccgcttcggggagaaccatgccatcatgggcgttgccttcacctgggtcatggcgctggcctgcgccgcacccccactcgccggctggtccaggtacatccccgagggcctgcagtgctcgtgtggaatcgactactacacgctcaagccggaggtcaacaacgagtcttttgtcatctacatgttcgtggtccacttcaccatccccatgattatcatctttttctgctatgggcagctcgtcttcaccgtcaaggaggccgctgcccagcagcaggagtcagccaccacacagaaggcagagaaggaggtcacccgcatggtcatcatcatggtcatcgctttcctgatctgctgggtgccctacgccagcgtggcattctacatcttcacccaccagggctccaacttcggtcccatcttcatgaccatcccagcgttctttgccaagagcgccgccatctacaaccctgtcatctatatcatgatgaacaagcagttccggaactgcatgctcaccaccatctgctgcggcaagaacccactgggtgacgatgaggcctctgctaccgtgtccaagacggagacgagccaggtggccccggcc

SEQ ID NO: 10 - DNA, 797 bp, Gallus gallus
  source 1..797: mol_type = other DNA
cgttacataacttacggtaaatggcccgcctggctgaccgcccaacgacccccgcccattgacgtcaatagtaacgccaatagggactttccattgacgtcaatgggtggagtatttacggtaaactgcccacttggcagtacatcaagtgtatcatatgccaagtacgccccctattgacgtcaatgacggtaaatggcccgcctggcattgtgcccagtacatgaccttatgggactttcctacttggcagtacatctacgtattagtcatcgctattaccatggtcgaggtgagccccacgttctgcttcactctccccatctcccccccctccccacccccaattttgtatttatttattttttaattattttgtgcagcgatgggggcggggggggggggggggcgcgcgccaggcggggcggggcggggcgaggggcggggcggggcgaggcggagaggtgcggcggcagccaatcagagcggcgcgctccgaaagtttccttttatggcgaggcggcggcggcggcggccctataaaaagcgaagcgcgcggcgggcgggagtcgctgcgacgctgccttcgccccgtgccccgctccgccgccgcctcgcgccgcccgccccggctctgactgaccgcgttactcccacaggtgagcgggcgggacggcccttctcctccgggctgtaattagctgagcaagaggtaagggtttaagggatggttggttggtggggtattaatgtttaattacctggagcacctgcctgaaatcactttttttcaggtt

SEQ ID NO: 11 - DNA, 232 bp, Bos taurus
  source 1..232: mol_type = other DNA
taagagctcgctgatcagcctcgactgtgccttctagttgccagccatctgttgtttgcccctcccccgtgccttccttgaccctggaaggtgccactcccactgtcctttcctaataaaatgaggaaattgcatcgcattgtctgagtaggtgtcattctattctggggggtggggtggggcaggacagcaagggggaggattgggaagagaatagcaggcatgctgggga

SEQ ID NO: 12 - DNA, 249 bp, Homo sapiens
  source 1..249: mol_type = other DNA
gagggcctatttcccatgattccttcatatttgcatatacgatacaaggctgttagagagataattggaattaatttgactgtaaacacaaagatattagtacaaaatacgtgacgtagaaagtaataatttcttgggtagtttgcagttttaaaattatgttttaaaatggactatcatatgcttaccgtaacttgaaagtatttcgatttcttggctttatatatcttgtggaaaggacgaaacacc

SEQ ID NO: 13 - DNA, 130 bp, Adeno-associated virus-2
  source 1..130: mol_type = other DNA
cgcgctcgctcgctcactgaggccgcccgggcaaagcccgggcgtcgggcgacctttggtcgcccggcctcagtgagcgagcgagcgcgcagagagggagtggccaactccatcactaggggttccttgt

SEQ ID NO: 14 - DNA, 173 bp, Human herpesvirus 5
  source 1..173: mol_type = other DNA
actcacggggatttccaagtctccaccccattgacgtcaatgggagtttgttttggcaccaaaatcaacgggactttccaaaatgtcgtaataaccccgccccgttgacgcaaatgggcggtaggcgtgtacggtgggaggtctatataagcagagctcgtttagtgaaccgt

SEQ ID NO: 15 - DNA, 66 bp, synthetic construct
  misc_feature 1..66: note = Description of Artificial Sequence: Synthetic oligonucleotide
  source 1..66: mol_type = other DNA
gactataaggaccacgacggagactacaaggatcatgatattgattacaaagacgatgacgataag

SEQ ID NO: 16 - DNA, 21 bp, Simian virus 40
  source 1..21: mol_type = other DNA
ccaaagaagaagcggaaggtc

SEQ ID NO: 17 - DNA, 4101 bp, Streptococcus pyogenes
  source 1..4101: mol_type = other DNA
gacaagaagtacagcatcggcctggacatcggcaccaactctgtgggctgggccgtgatcaccgacgagtacaaggtgcccagcaagaaattcaaggtgctgggcaacaccgaccggcacagcatcaagaagaacctgatcggagccctgctgttcgacagcggcgaaacagccgaggccacccggctgaagagaaccgccagaagaagatacaccagacggaagaaccggatctgctatctgcaagagatcttcagcaacgagatggccaaggtggacgacagcttcttccacagactggaagagtccttcctggtggaagaggataagaagcacgagcggcaccccatcttcggcaacatcgtggacgaggtggcctaccacgagaagtaccccaccatctaccacctgagaaagaaactggtggacagcaccgacaaggccgacctgcggctgatctatctggccctggcccacatgatcaagttccggggccacttcctgatcgagggcgacctgaaccccgacaacagcgacgtggacaagctgttcatccagctggtgcagacctacaaccagctgttcgaggaaaaccccatcaacgccagcggcgtggacgccaaggccatcctgtctgccagactgagcaagagcagacggctggaaaatctgatcgcccagctgcccggcgagaagaagaatggcctgttcggaaacctgattgccctgagcctgggcctgacccccaacttcaagagcaacttcgacctggccgaggatgccaaactgcagctgagcaaggacacctacgacgacgacctggacaacctgctggcccagatcggcgaccagtacgccgacctgtttctggccgccaagaacctgtccgacgccatcctgctgagcgacatcctgagagtgaacaccgagatcaccaaggcccccctgagcgcctctatgatcaagagatacgacgagcaccaccaggacctgaccctgctgaaagctctcgtgcggcagcagctgcctgagaagtacaaagagattttcttcgaccagagcaagaacggctacgccggctacattgacggcggagccagccaggaagagttctacaagttcatcaagcccatcctggaaaagatggacggcaccgaggaactgctcgtgaagctgaacagagaggacctgctgcggaagcagcggaccttcgacaacggcagcatcccccaccagatccacctgggagagctgcacgccattctgcggcggcaggaagatttttacccattcctgaaggacaaccgggaaaagatcgagaagatcctgaccttccgcatcccctactacgtgggccctctggccaggggaaacagcagattcgcctggatgaccagaaagagcgaggaaaccatcaccccctggaacttcgaggaagtggtggacaagggcgcttccgcccagagcttcatcgagcggatgaccaacttcgataagaacctgcccaacgagaaggtgctgcccaagcacagcctgctgtacgagtacttcaccgtgtataacgagctgaccaaagtgaaatacgtgaccgagggaatgagaaagcccgccttcctgagcggcgagcagaaaaaggccatcgtggacctgctgttcaagaccaaccggaaagtgaccgtgaagcagctgaaagaggactacttcaagaaaatcgagtgcttcgactccgtggaaatctccggcgtggaagatcggttcaacgcctccctgggcacataccacgatctgctgaaaattatcaaggacaaggacttcctggacaatgaggaaaacgaggacattctggaagatatcgtgctgaccctgacactgtttgaggacagagagatgatcgaggaacggctgaaaacctatgcccacctgttcgacgacaaagtgatgaagcagctgaagcggcggagatacaccggctggggcaggctgagccggaagctgatcaacggcatccgggacaagcagtccggcaagacaatcctggatttcctgaagtccgacggcttcgccaacagaaacttcatgcagctgatccacgacgacagcctgacctttaaagaggacatccagaaagcccaggtgtccggccagggcgatagcctgcacgagcacattgccaatctggccggcagccccgccattaagaagggcatcctgcagacagtgaaggtggtggacgagctcgtgaaagtgatgggccggcacaagcccgagaacatcgtgatcgaaatggccagagagaaccagaccacccagaagggacagaagaacagccgcgagagaatgaagcggatcgaagagggcatcaaagagctgggcagccagatcctgaaagaacaccccgtggaaaacacccagctgcagaacgagaagctgtacctgtactacctgcagaatgggcgggatatgtacgtggaccaggaactggacatcaaccggctgtccgactacgatgtggaccatatcgtgcctcagagctttctgaaggacgactccatcgacaacaaggtgctgaccagaagcgacaagaaccggggcaagagcgacaacgtgccctccgaagaggtcgtgaagaagatgaagaactactggcggcagctgctgaacgccaagctgattacccagagaaagttcgacaatctgaccaaggccgagagaggcggcctgagcgaactggataaggccggcttcatcaagagacagctggtggaaacccggcagatcacaaagcacgtggcacagatcctggactcccggatgaacactaagtacgacgagaatgacaagctgatccgggaagtgaaagtgatcaccctgaagtccaagctggtgtccgatttccggaaggatttccagttttacaaagtgcgcgagatcaacaactaccaccacgcccacgacgcctacctgaacgccgtcgtgggaaccgccctgatcaaaaagtaccctaagctggaaagcgagttcgtgtacggcgactacaaggtgtacgacgtgcggaagatgatcgccaagagcgagcaggaaatcggcaaggctaccgccaagtacttcttctacagcaacatcatgaactttttcaagaccgagattaccctggccaacggcgagatccggaagcggcctctgatcgagacaaacggcgaaaccggggagatcgtgtgggataagggccgggattttgccaccgtgcggaaagtgctgagcatgccccaagtgaatatcgtgaaaaagaccgaggtgcagacaggcggcttcagcaaagagtctatcctgcccaagaggaacagcgataagctgatcgccagaaagaaggactgggaccctaagaagtacggcggcttcgacagccccaccgtggcctattctgtgctggtggtggccaaagtggaaaagggcaagtccaagaaactgaagagtgtgaaagagctgctggggatcaccatcatggaaagaagcagcttcgagaagaatcccatcgactttctggaagccaagggctacaaagaagtgaaaaaggacctgatcatcaagctgcctaagtactccctgttcgagctggaaaacggccggaagagaatgctggcctctgccggcgaactgcagaagggaaacgaactggccctgccctccaaatatgtgaacttcctgtacctggccagccactatgagaagctgaagggctcccccgaggataatgagcagaaacagctgtttgtggaacagcacaagcactacctggacgagatcatcgagcagatcagcgagttctccaagagagtgatcctggccgacgctaatctggacaaagtgctgtccgcctacaacaagcaccgggataagcccatcagagagcaggccgagaatatcatccacctgtttaccctgaccaatctgggagcccctgccgccttcaagtactttgacaccaccatcgaccggaagaggtacaccagcaccaaagaggtgctggacgccaccctgatccaccagagcatcaccggcctgtacgagacacggatcgacctgtctcagctgggaggcgac

SEQ ID NO: 18 - DNA, 48 bp, Xenopus laevis
  source 1..48: mol_type = other DNA
aaaaggccggcggccacgaaaaaggccggccaggcaaaaaagaaaaag

SEQ ID NO: 19 - DNA, 49 bp, Oryctolagus cuniculus
  source 1..49: mol_type = other DNA
aataaaagatctttattttcattagatctgtgtgttggttttttgtgtg

SEQ ID NO: 20 - DNA, 508 bp, Human herpesvirus 5
  source 1..508: mol_type = other DNA
cgttacataacttacggtaaatggcccgcctggctgaccgcccaacgacccccgcccattgacgtcaataatgacgtatgttcccatagtaacgccaatagggactttccattgacgtcaatgggtggagtatttacggtaaactgcccacttggcagtacatcaagtgtatcatatgccaagtacgccccctattgacgtcaatgacggtaaatggcccgcctggcattatgcccagtacatgaccttatgggactttcctacttggcagtacatctacgtattagtcatcgctattaccatggtgatgcggttttggcagtacatcaatgggcgtggatagcggtttgactcacggggatttccaagtctccaccccattgacgtcaatgggagtttgttttggcaccaaaatcaacgggactttccaaaatgtcgtaacaactccgccccattgacgcaaatgggcggtaggcgtgtacggtgggaggtctatataagcagagct

SEQ ID NO: 21 - DNA, 720 bp, Aequorea victoria
  source 1..720: mol_type = other DNA
atggtgagcaagggcgaggagctgttcaccggggtggtgcccatcctggtcgagctggacggcgacgtaaacggccacaagttcagcgtgtccggcgagggcgagggcgatgccacctacggcaagctgaccctgaagttcatctgcaccaccggcaagctgcccgtgccctggcccaccctcgtgaccaccctgacctacggcgtgcagtgcttcagccgctaccccgaccacatgaagcagcacgacttcttcaagtccgccatgcccgaaggctacgtccaggagcgcaccatcttcttcaaggacgacggcaactacaagacccgcgccgaggtgaagttcgagggcgacaccctggtgaaccgcatcgagctgaagggcatcgacttcaaggaggacggcaacatcctggggcacaagctggagtacaactacaacagccacaacgtctatatcatggccgacaagcagaagaacggcatcaaggtgaacttcaagatccgccacaacatcgaggacggcagcgtgcagctcgccgaccactaccagcagaacacccccatcggcgacggccccgtgctgctgcccgacaaccactacctgagcacccagtccgccctgagcaaagaccccaacgagaagcgcgatcacatggtcctgctggagttcgtgaccgccgccgggatcactctcggcatggacgagctgtacaagtaa

SEQ ID NO: 22 - DNA, 9175 bp, Streptococcus pyogenes
  source 1..9175: mol_type = other DNA
gagggcctatttcccatgattccttcatatttgcatatacgatacaaggctgttagagagataattggaattaatttgactgtaaacacaaagatattagtacaaaatacgtgacgtagaaagtaataatttcttgggtagtttgcagttttaaaattatgttttaaaatggactatcatatgcttaccgtaacttgaaagtatttcgatttcttggctttatatatcttgtggaaaggacgaaacaccgggtcttcgagaagacctgttttagagctagaaatagcaagttaaaataaggctagtccgttatcaacttgaaaaagtggcaccgagtcggtgcttttttgttttagagctagaaatagcaagttaaaataaggctagtccgtttttagcgcgtgcgccaattctgcagacaaatggctctagaggtacccgttacataacttacggtaaatggcccgcctggctgaccgcccaacgacccccgcccattgacgtcaatagtaacgccaatagggactttccattgacgtcaatgggtggagtatttacggtaaactgcccacttggcagtacatcaagtgtatcatatgccaagtacgccccctattgacgtcaatgacggtaaatggcccgcctggcattgtgcccagtacatgaccttatgggactttcctacttggcagtacatctacgtattagtcatcgctattaccatggtcgaggtgagccccacgttctgcttcactctccccatctcccccccctccccacccccaattttgtatttatttattttttaattattttgtgcagcgatgggggcggggggggggggggggcgcgcgccaggcggggcggggcggggcgaggggcggggcggggcgaggcggagaggtgcggcggcagccaatcagagcggcgcgctccgaaagtttccttttatggcgaggcggcggcggcggcggccctataaaaagcgaagcgcgcggcgggcgggagtcgctgcgacgctgccttcgccccgtgccccgctccgccgccgcctcgcgccgcccgccccggctctgactgaccgcgttactcccacaggtgagcgggcgggacggcccttctcctccgggctgtaattagctgagcaagaggtaagggtttaagggatggttggttggtggggtattaatgtttaattacctggagcacctgcctgaaatcactttttttcaggttggaccggtgccaccatggactataaggaccacgacggagactacaaggatcatgatattgattacaaagacgatgacgataagatggccccaaagaagaagcggaaggtcggtatccacggagtcccagcagccgacaagaagtacagcatcggcctggacatcggcaccaactctgtgggctgggccgtgatcaccgacgagtacaaggtgcccagcaagaaattcaaggtgctgggcaacaccgaccggcacagcatcaagaagaacctgatcggagccctgctgttcgacagcggcgaaacagccgaggccacccggctgaagagaaccgccagaagaagatacaccagacggaagaaccggatctgctatctgcaagagatcttcagcaacgagatggccaaggtggacgacagcttcttccacagactggaagagtccttcctggtggaagaggataagaagcacgagcggcaccccatcttcggcaacatcgtggacgaggtggcctaccacgagaagtaccccaccatctaccacctgagaaagaaactggtggacagcaccgacaaggccgacctgcggctgatctatctggccctggcccacatgatcaagttccggggccacttcctgatcgagggcgacctgaaccccgacaacagcgacgtggacaagctgttcatccagctggtgcagacctacaaccagctgttcgaggaaaaccccatcaacgccagcggcgtggacgccaaggccatcctgtctgccagactgagcaagagcagacggctggaaaatctgatcgcccagctgcccggcgagaagaagaatggcctgttcggaaacctgattgccctgagcctgggcctgacccccaacttcaagagcaacttcgacctggccgaggatgccaaactgcagctgagcaaggacacctacgacgacgacctggacaacctgctggcccagatcggcgaccagtacgccgacctgtttctggccgccaagaacctgtccgacgccatcctgctgagcgacatcctgagagtgaacaccgagatcaccaaggcccccctgagcgcctctatgatcaagagatacgacgagcaccaccaggacctgaccctgctgaaagctctcgtgcggcagcagctgcctgagaagtacaaagagattttcttcgaccagagcaagaacggctacgccggctacattgacggcggagccagccaggaagagttctacaagttcatcaagcccatcctggaaaagatggacggcaccgaggaactgctcgtgaagctgaacagagaggacctgctgcggaagcagcggaccttcgacaacggcagcatcccccaccagatccacctgggagagctgcacgccattctgcggcggcaggaagatttttacccattcctgaaggacaaccgggaaaagatcgagaagatcctgaccttccgcatcccctactacgtgggccctctggccaggggaaacagcagattcgcctggatgaccagaaagagcgaggaaaccatcaccccctggaacttcgaggaagtggtggacaagggcgcttccgcccagagcttcatcgagcggatgaccaacttcgataagaacctgcccaacgagaaggtgctgcccaagcacagcctgctgtacgagtacttcaccgtgtataacgagctgaccaaagtgaaatacgtgaccgagggaatgagaaagcccgccttcctgagcggcgagcagaaaaaggccatcgtggacctgctgttcaagaccaaccggaaagtgaccgtgaagcagctgaaagaggactacttcaagaaaatcgagtgcttcgactccgtggaaatctccggcgtggaagatcggttcaacgcctccctgggcacataccacgatctgctgaaaattatcaaggacaaggacttcctggacaatgaggaaaacgaggacattctggaagatatcgtgctgaccctgacactgtttgaggacagagagatgatcgaggaacggctgaaaacctatgcccacctgttcgacgacaaagtgatgaagcagctgaagcggcggagatacaccggctggggcaggctgagccggaagctgatcaacggcatccgggacaagcagtccggcaagacaatcctggatttcctgaagtccgacggcttcgccaacagaaacttcatgcagctgatccacgacgacagcctgacctttaaagaggacatccagaaagcccaggtgtccggccagggcgatagcctgcacgagcacattgccaatctggccggcagccccgccattaagaagggcatcctgcagacagtgaaggtggtggacgagctcgtgaaagtgatgggccggcacaagcccgagaacatcgtgatcgaaatggccagagagaaccagaccacccagaagggacagaagaacagccgcgagagaatgaagcggatcgaagagggcatcaaagagctgggcagccagatcctgaaagaacaccccgtggaaaacacccagctgcagaacgagaagctgtacctgtactacctgcagaatgggcgggatatgtacgtggaccaggaactggacatcaaccggctgtccgactacgatgtggaccatatcgtgcctcagagctttctgaaggacgactccatcgacaacaaggtgctgaccagaagcgacaagaaccggggcaagagcgacaacgtgccctccgaagaggtcgtgaagaagatgaagaactactggcggcagctgctgaacgccaagctgattacccagagaaagttcgacaatctgaccaaggccgagagaggcggcctgagcgaactggataaggccggcttcatcaagagacagctggtggaaacccggcagatcacaaagcacgtggcacagatcctggactcccggatgaacactaagtacgacgagaatgacaagctgatccgggaagtgaaagtgatcaccctgaagtccaagctggtgtccgatttccggaaggatttccagttttacaaagtgcgcgagatcaacaactaccaccacgcccacgacgcctacctgaacgccgtcgtgggaaccgccctgatcaaaaagtaccctaagctggaaagcgagttcgtgtacggcgactacaaggtgtacgacgtgcggaagatgatcgccaagagcgagcaggaaatcggcaaggctaccgccaagtacttcttctacagcaacatcatgaactttttcaagaccgagattaccctggccaacggcgagatccggaagcggcctctgatcgagacaaacggcgaaaccggggagatcgtgtgggataagggccgggattttgccaccgtgcggaaagtgctgagcatgccccaagtgaatatcgtgaaaaagaccgaggtgcagacaggcggcttcagcaaagagtctatcctgcccaagaggaacagcgataagctgatcgccagaaagaaggactgggaccctaagaagtacggcggcttcgacagccccaccgtggcctattctgtgctggtggtggccaaagtggaaaagggcaagtccaagaaactgaagagtgtgaaagagctgctggggatcaccatcatggaaagaagcagcttcgagaagaatcccatcgactttctggaagccaagggctacaaagaagtgaaaaaggacctgatcatcaagctgcctaagtactccctgttcgagctggaaaacggccggaagagaatgctggcctctgccggcgaactgcagaagggaaacgaactggccctgccctccaaatatgtgaacttcctgtacctggccagccactatgagaagctgaagggctcccccgaggataatgagcagaaacagctgtttgtggaacagcacaagcactacctggacgagatcatcgagcagatcagcgagttctccaagagagtgatcctggccgacgctaatctggacaaagtgctgtccgcctacaacaagcaccgggataagcccatcagagagcaggccgagaatatcatccacctgtttaccctgaccaatctgggagcccctgccgccttcaagtactttgacaccaccatcgaccggaagaggtacaccagcaccaaagaggtgctggacgccaccctgatccaccagagcatcaccggcctgtacgagacacggatcgacctgtctcagctgggaggcgacaaaaggccggcggccacgaaaaaggccggccaggcaaaaaagaaaaaggaattcggcagtggagagggcagaggaagtctgctaacatgcggtgacgtcgaggagaatcctggcccaatgaccgagtacaagcccacggtgcgcctcgccacccgcgacgacgtccccagggccgtacgcaccctcgccgccgcgttcgccgactaccccgccacgcgccacaccgtcgatccggaccgccacatcgagcgggtcaccgagctgcaagaactcttcctcacgcgcgtcgggctcgacatcggcaaggtgtgggtcgcggacgacggcgccgcggtggcggtctggaccacgccggagagcgtcgaagcgggggcggtgttcgccgagatcggcccgcgcatggccgagttgagcggttcccggctggccgcgcagcaacagatggaaggcctcctggcgccgcaccggcccaaggagcccgcgtggttcctggccaccgtcggagtctcgcccgaccaccagggcaagggtctgggcagcgccgtcgtgctccccggagtggaggcggccgagcgcgccggggtgcccgccttcctggagacctccgcgccccgcaacctccccttctacgagcggctcggcttcaccgtcaccgccgacgtcgaggtgcccgaaggaccgcgcacctggtgcatgacccgcaagcccggtgcctgagaattctaactagagctcgctgatcagcctcgactgtgccttctagttgccagccatctgttgtttgcccctcccccgtgccttccttgaccctggaaggtgccactcccactgtcctttcctaataaaatgaggaaattgcatcgcattgtctgagtaggtgtcattctattctggggggtggggtggggcaggacagcaagggggaggattgggaagagaatagcaggcatgctggggagcggccgcaggaacccctagtgatggagttggccactccctctctgcgcgctcgctcgctcactgaggccgggcgaccaaaggtcgcccgacgcccgggctttgcccgggcggcctcagtgagcgagcgagcgcgcagctgcctgcaggggcgcctgatgcggtattttctccttacgcatctgtgcggtatttcacaccgcatacgtcaaagcaaccatagtacgcgccctgtagcggcgcattaagcgcggcgggtgtggtggttacgcgcagcgtgaccgctacacttgccagcgccctagcgcccgctcctttcgctttcttcccttcctttctcgccacgttcgccggctttccccgtcaagctctaaatcgggggctccctttagggttccgatttagtgctttacggcacctcgaccccaaaaaacttgatttgggtgatggttcacgtagtgggccatcgccctgatagacggtttttcgccctttgacgttggagtccacgttctttaatagtggactcttgttccaaactggaacaacactcaaccctatctcgggctattcttttgatttataagggattttgccgatttcggcctattggttaaaaaatgagctgatttaacaaaaatttaacgcgaattttaacaaaatattaacgtttacaattttatggtgcactctcagtacaatctgctctgatgccgcatagttaagccagccccgacacccgccaacacccgctgacgcgccctgacgggcttgtctgctcccggcatccgcttacagacaagctgtgaccgtctccgggagctgcatgtgtcagaggttttcaccgtcatcaccgaaacgcgcgagacgaaagggcctcgtgatacgcctatttttataggttaatgtcatgataataatggtttcttagacgtcaggtggcacttttcggggaaatgtgcgcggaacccctatttgtttatttttctaaatacattcaaatatgtatccgctcatgagacaataaccctgataaatgcttcaataatattgaaaaaggaagagtatgagtattcaacatttccgtgtcgcccttattcccttttttgcggcattttgccttcctgtttttgctcacccagaaacgctggtgaaagtaaaagatgctgaagatcagttgggtgcacgagtgggttacatcgaactggatctcaacagcggtaagatccttgagagttttcgccccgaagaacgttttccaatgatgagcacttttaaagttctgctatgtggcgcggtattatcccgtattgacgccgggcaagagcaactcggtcgccgcatacactattctcagaatgacttggttgagtactcaccagtcacagaaaagcatcttacggatggcatgacagtaagagaattatgcagtgctgccataaccatgagtgataacactgcggccaacttacttctgacaacgatcggaggaccgaaggagctaaccgcttttttgcacaacatgggggatcatgtaactcgccttgatcgttgggaaccggagctgaatgaagccataccaaacgacgagcgtgacaccacgatgcctgtagcaatggcaacaacgttgcgcaaactattaactggcgaactacttactctagcttcccggcaacaattaatagactggatggaggcggataaagttgcaggaccacttctgcgctcggcccttccggctggctggtttattgctgataaatctggagccggtgagcgtggaagccgcggtatcattgcagcactggggccagatggtaagccctcccgtatcgtagttatctacacgacggggagtcaggcaactatggatgaacgaaatagacagatcgctgagataggtgcctcactgattaagcattggtaactgtcagaccaagtttactcatatatactttagattgatttaaaacttcatttttaatttaaaaggatctaggtgaagatcctttttgataatctcatgaccaaaatcccttaacgtgagttttcgttccactgagcgtcagaccccgtagaaaagatcaaaggatcttcttgagatcctttttttctgcgcgtaatctgctgcttgcaaacaaaaaaaccaccgctaccagcggtggtttgtttgccggatcaagagctaccaactctttttccgaaggtaactggcttcagcagagcgcagataccaaatactgtccttctagtgtagccgtagttaggccaccacttcaagaactctgtagcaccgcctacatacctcgctctgctaatcctgttaccagtggctgctgccagtggcgataagtcgtgtcttaccgggttggactcaagacgatagttaccggataaggcgcagcggtcgggctgaacggggggttcgtgcacacagcccagcttggagcgaacgacctacaccgaactgagatacctacagcgtgagctatgagaaagcgccacgcttcccgaagggagaaaggcggacaggtatccggtaagcggcagggtcggaacaggagagcgcacgagggagcttccagggggaaacgcctggtatctttatagtcctgtcgggtttcgccacctctgacttgagcgtcgatttttgtgatgctcgtcaggggggcggagcctatggaaaaacgccagcaacgcggcctttttacggttcctggccttttgctggccttttgctcacatgt

SEQ ID NO: 23 - DNA, 380 bp, Mus musculus
  source 1..380: mol_type = other DNA
tcccttaaccaccgaaggcagggcagcaggctagtggagcagagctgcgtggtcaagtggcagggagcttaagaatcgtccaagggcggagaccagtaagtctcattaggtgatggggccagcaggtaaaagccattcatgcttatgtccagctgggcgtgtgttctcttcctgttttatcatcccttgcgctgaccatcaggtacatccctgagggcatgcaatgttcatgcgggattgactattatacccttaagccggaggtcaacaacgaatcctttgtcatctacatgttcgtggtccacttcaccattcctatgatcgtcatcttcttctgctatgggcagctggtcttcacagtcaaggaggtatgagcaggg

SEQ ID NO: 24 - DNA, 1958 bp, unidentified
  misc_feature 1..1958: note = Description of Unknown: Mouse or Human polynucleotide
  source 1..1958: mol_type = other DNA
atgctcacctgaataacctggcagcctgctccctcatgcagggaccacgtcctgctgcacccagcaggccatcccgtctccatagcccatggtcatccctccctggacaggaatgtgtctcctccccgggctgagtcttgctcaagctagaagcactccgaacagggttatgggcgcctcctccatctcccaagtggctggcttatgaatgtttaatgtacatgtgagtgaacaaattccaattgaacgcaacaaatagttatcgagccgctgagccggggggcggggggtgtgagactggaggcgatggacggagctgacggcacacacagctcagatctgtcaagtgagccattgtcagggcttggggactggataagtcagggggtctcctgggaagagatgggataggtgagttcaggaggagacattgtcaactggagccatgtggagaagtgaatttagggcccaaaggttccagtcgcagcctgaggccaccagactgacatggggaggaattcccagaggactctggggcagacaagatgagacaccctttcctttctttacctaagggcctccacccgatgtcaccttggcccctctgcaagccaattaggccccggtggcagcagtgggattagcgttagtatgatatctcgcggatgctgaatcagcctctggcttagggagagaaggtcactttataagggtctggggggggtcagtgcctggagttgcgctgtgggagcgagtcatccagctggagccctgagtggctgagctcaggccttcgcagcattcttgggtgggagcagccacgggtcagccacaagggccacagccatgaatggcacagaaggccctaacttctacgtgcccttctccaatgcgacgggtgtggtacgcagccccttcgagtacccacagtactacctggctgagccatggcagttctccatgctggccgcctacatgtttctgctgatcgtgctgggcttccccatcaacttcctcacgctctacgtcaccgtccagcacaagaagctgcgcacgcctctcaactacatcctgctcaacctagccgtggctgacctcttcatggtcctaggtggcttcaccagcaccctctacacctctctgcatggatacttcgtcttcgggcccacaggatgcaatttggagggcttctttgccaccctgggcggtatgagcagagagactggggcgggggggtgtagcatgggagccaaggggccacgaaagggcctgggagggtctgcagcttacttgagtctctttaattggtctcatctaaaggcccagcttattcattggcaaacactgtgaccctgagctaggctgctgttgagagcaggcacggaacattcatctatctcatcttgagcaatgcaagaaacatgggttcagagaggccaaggactcaccgaggagtcacagagtgtgggggtgtcctctgaggcagctgagctggggcacacacagactgagcaccaggagtgagctctagcttttttttttctatgtgtcttttctaaaagacacataggtttaggactgtccctggtccaggtaagaactggttcagtaaacttgtacatctcactgcctggccagccctgtcagcttccaccagagtgcgtgcactacacacccggcatctcaaaggattcattcctatctttcctatctttggagtgaggcacagtctcacgtagtccagtccagactggccttaaattctgcagctgaggatgtacttaaacttgtcatcctcctgccccagcctctcaagtgctgtgatcacaggcacggaccactatgctacgccaggtgtttccaaacattttctctcccttaactggaaggtcaatgaggctctttcgagaagcaacagagcctgtttagctgagaaaactgaggcagggagcaggcaa

SEQ ID NO: 25 - DNA, 1958 bp, unidentified
  misc_feature 1..1958: note = Description of Unknown: Mouse or Human polynucleotide
  source 1..1958: mol_type = other DNA
atgctcacctgaataacctggcagcctgctccctcatgcagggaccacgtcctgctgcacccagcaggccatcccgtctccatagcccatggtcatccctccctggacaggaatgtgtctcctccccgggctgagtcttgctcaagctagaagcactccgaacagggttatgggcgcctcctccatctcccaagtggctggcttatgaatgtttaatgtacatgtgagtgaacaaattccaattgaacgcaacaaatagttatcgagccgctgagccggggggcggggggtgtgagactggaggcgatggacggagctgacggcacacacagctcagatctgtcaagtgagccattgtcagggcttggggactggataagtcagggggtctcctgggaagagatgggataggtgagttcaggaggagacattgtcaactggagccatgtggagaagtgaatttagggcccaaaggttccagtcgcagcctgaggccaccagactgacatggggaggaattcccagaggactctggggcagacaagatgagacaccctttcctttctttacctaagggcctccacccgatgtcaccttggcccctctgcaagccaattaggccccggtggcagcagtgggattagcgttagtatgatatctcgcggatgctgaatcagcctctggcttagggagagaaggtcactttataagggtctggggggggtcagtgcctggagttgcgctgtgggagcgagtcatccagctggagccctgagtggctgagctcaggccttcgcagcattcttgggtgggagcagccacgggtcagccacaagggccacagccatgaatggcacagaaggccctaacttctacgtgcccttctccaatgcgacgggtgtggtacgcagccccttcgagtacccacagtactacctggctgagccatggcagttctccatgctggccgcctacatgtttctgctgatcgtgctgggcttccccatcaacttcctcacgctctacgtcaccgtccagcacaagaagctgcgcacgcctctcaactacatcctgctcaacctagccgtggctgacctcttcatggtcctaggtggcttcaccagcaccctctacacctctctgcatggatacttcgtcttcgggcccacaggacgcaatttggagggcttctttgccaccctgggcggtatgagcagagagactggggcgggggggtgtagcatgggagccaaggggccacgaaagggcctgggagggtctgcagcttacttgagtctctttaattggtctcatctaaaggcccagcttattcattggcaaacactgtgaccctgagctaggctgctgttgagagcaggcacggaacattcatctatctcatcttgagcaatgcaagaaacatgggttcagagaggccaaggactcaccgaggagtcacagagtgtgggggtgtcctctgaggcagctgagctggggcacacacagactgagcaccaggagtgagctctagcttttttttttctatgtgtcttttctaaaagacacataggtttaggactgtccctggtccaggtaagaactggttcagtaaacttgtacatctcactgcctggccagccctgtcagcttccaccagagtgcgtgcactacacacccggcatctcaaaggattcattcctatctttcctatctttggagtgaggcacagtctcacgtagtccagtccagactggccttaaattctgcagctgaggatgtacttaaacttgtcatcctcctgccccagcctctcaagtgctgtgatcacaggcacggaccactatgctacgccaggtgtttccaaacattttctctcccttaactggaaggtcaatgaggctctttcgagaagcaacagagcctgtttagctgagaaaactgaggcagggagcaggcaa

SEQ ID NO: 26 - DNA, 469 bp, Mus musculus
  source 1..469: mol_type = other DNA
tgagagatgaggtagggtggcgcccatctcgagggcagcttgcgtgagcacaggcagccttcttgccattggctgaggctgtcattgccgtcaccacttcgggtgggcaccggaagaagagtgaccttattgccagcaccatttctcaaacgttgtctaattcttttctctagagcctgaatatcttccagaatctcaaccgacgtcaacacgagcatgcgatccacatgatggacatcgcgatcattgccacagaccttgccttgtatttcaagtgggtatttctcctcactttaatagtagcagtgtgggggctggagagatggttcagtggttaacagcactgactgctcttccagaggtcctgagttcaaatcccagcaaccacatggtggctcacaactatctgtaatgggatctgataccctcttctggtgtgtgtctgaagacagcgatggagtactcacat

SEQ ID NO: 27 - DNA, 128 bp, Homo sapiens
  source 1..128: mol_type = other DNA
tagttagtaaactctttgaccctacatctctacagatataaatgagtgtgagaccacaaacgagtgccgggaggatgaaatgtgttggaattatcatggcggcttccgttgttatccacgaaatcctt

SEQ ID NO: 28 - DNA, 19 bp, Homo sapiens
  source 1..19: mol_type = other DNA
ccttcgtccagccgcagag

SEQ ID NO: 29 - DNA, 13 bp, Homo sapiens
  source 1..13: mol_type = other DNA
tggaagggtaggt

SEQ ID NO: 30 - DNA, 36 bp, Homo sapiens
  source 1..36: mol_type = other DNA
gaggagctgaaacctactgtagggaaaggtgcggac

SEQ ID NO: 31 - DNA, 21 bp, Homo sapiens
  source 1..21: mol_type = other DNA
agaggagctgaaacctacccg

SEQ ID NO: 32 - DNA, 28 bp, Homo sapiens
  source 1..28: mol_type = other DNA
gagaggagctgaaacctacccggggtca

SEQ ID NO: 33 - DNA, 28 bp, Homo sapiens
  source 1..28: mol_type = other DNA
ctctcctcgactttggatgggccccagt

SEQ ID NO: 34 - DNA, 20 bp, synthetic construct
  misc_feature 1..20: note = Synthetic
  source 1..20: mol_type = other DNA
cacagccaggaatggaccat

SEQ ID NO: 35 - DNA, 20 bp, synthetic construct
  misc_feature 1..20: note = Synthetic
  source 1..20: mol_type = other DNA
atggtccattcctggctgtg

SEQ ID NO: 36 - DNA, 20 bp, synthetic construct
  misc_feature 1..20: note = Synthetic
  source 1..20: mol_type = other DNA
taagtgtgcaagtcagaaca

SEQ ID NO: 37 - DNA, 20 bp, synthetic construct
  misc_feature 1..20: note = Synthetic
  source 1..20: mol_type = other DNA
cagcagctgaggtttaaagg

SEQ ID NO: 38 - DNA, 20 bp, synthetic construct
  misc_feature 1..20: note = Synthetic
  source 1..20: mol_type = other DNA
gtctgaggctgagtatcggg

SEQ ID NO: 39 - DNA, 20 bp, synthetic construct
  misc_feature 1..20: note = Synthetic
  source 1..20: mol_type = other DNA
ggtctcgctatgttgctcag

SEQ ID NO: 40 - DNA, 20 bp, synthetic construct
  misc_feature 1..20: note = Synthetic
  source 1..20: mol_type = other DNA
agaggagctgaaacctaccc

SEQ ID NO: 41 - DNA, 20 bp, synthetic construct
  misc_feature 1..20: note = Synthetic
  source 1..20: mol_type = other DNA
gaggagctgaaacctacccg

SEQ ID NO: 42 - DNA, 20 bp, synthetic construct
  misc_feature 1..20: note = Synthetic
  source 1..20: mol_type = other DNA
ccacaaaggagtccttgtct

SEQ ID NO: 43 - DNA, 20 bp, synthetic construct
  misc_feature 1..20: note = Synthetic
  source 1..20: mol_type = other DNA
ttagagtagttttaggttca

SEQ ID NO: 44 - DNA, 20 bp, synthetic construct
  misc_feature 1..20: note = Synthetic
  source 1..20: mol_type = other DNA
ttcttgggtgggagcagcca

SEQ ID NO: 45 - DNA, 20 bp, synthetic construct
  misc_feature 1..20: note = Synthetic
  source 1..20: mol_type = other DNA
ttcttgggtgggagcagccg

SEQ ID NO: 46 - DNA, 20 bp, synthetic construct
  misc_feature 1..20: note = Synthetic
  source 1..20: mol_type = other DNA
tgaaggccaagttcccaatg

SEQ ID NO: 47 - DNA, 20 bp, synthetic construct
  misc_feature 1..20: note = Synthetic
  source 1..20: mol_type = other DNA
tgaaggccaagttcccagtg

SEQ ID NO: 48 - DNA, 20 bp, synthetic construct
  misc_feature 1..20: note = Synthetic
  source 1..20: mol_type = other DNA
ggacggtgacgtagagcgtg

SEQ ID NO: 49 - DNA, 20 bp, synthetic construct
  misc_feature 1..20: note = Synthetic
  source 1..20: mol_type = other DNA
gacgaagtatccatgcagag